European Patent Specification EP 3 507 371 B1, published January 28, 2026. Title: METHODS AND COMPOSITIONS FOR TREATING DISEASES AND DISORDERS OF THE NERVOUS SYSTEM. Applicant: Rutgers, The State University of New Jersey Bowery, Hannah E. Aston-Jones, Gary. The sequence listing filed with the application follows.

SEQUENCE LISTING (11 sequences)

SEQ ID NO: 1 - DNA, 4711 bp, Artificial Sequence
  PACAP- hM3D(Gq)-mCherry Construct
caatcttaaattttcaattattgcagaaaacacagtgacatggtttcaatttttaaaactagtaagagccacggagagtgtgaaagtgtgtagacaggaaaggtaaagatccatctgaatactaggactaactcagaagaaaaagctttgcactgaggcagggattaagcaggttctgagcactgggacattcgtggacacagaatccaagggaagattaatatgaacagcggggtgatttagacaatgaactcccacagtaagagcaccactgccaaagcttcaaatttagaggctgtggtgaaaattaaaccagtggcaaatttcaacatttgcagcatctgcgcccaaatagttcagcaccaagagcctggacagcaccacaggctctcatcctagtctcatccatcaatctattcagagacagactgtcaacccagccagactcattagatatttactgaaaatccttataattctttcctttaaaacacaaaacgacttccatgtttagtagcctatttgaaaaagcatatgcaaggaattgagagatcaaaattaaaattattaataggagatcttgatggtgcttaaatctagagatcagagttgtcattggtgggggttgagtgaaaattaagaaaaattagggactcaataaaaacatgacttcaccattctctaaattctacgagttctttacttgtctttgagaaatcagtgaaatcgaaaaccatcaaaataattggacttcttaaaaattggattgtgtgagtgaaaggtgtttatcagaagcggatgactccggatcttatcatcctggaggactgcacagaatagttaatatgttccttgagggactaggatgctgacgtcttttactgataccggatcattacgtgactgggggagaaaaaaaaggaagtcatatcatgaataaaaatcggagtgcaacagtgcaaccaaaatattctgtacttgaaggcagaaagatgttgacaaagaggtgtctcctgaaaccacgttcggacagcttattttgttaactgcatatataaaaacgagcagaaggccagtgtcgacgccaccatgaccttgcacaataacagtacaacctcgcctttgtttccaaacatcagctcctcctggatacacagcccctccgatgcagggctgcccccgggaaccgtcactcatttcggcagctacaatgtttctcgagcagctggcaatttctcctctccagacggtaccaccgatgaccctctgggaggtcataccgtctggcaagtggtcttcatcgctttcttaacgggcatcctggccttggtgaccatcatcggcaacatcctggtaattgtgtcatttaaggtcaacaagcagctgaagacggtcaacaactacttcctcttaagcctggcctgtgccgatctgattatcggggtcatttcaatgaatctgtttacgacctacatcatcatgaatcgatgggccttagggaacttggcctgtgacctctggcttgccattgactgcgtagccagcaatgcctctgttatgaatcttctggtcatcagctttgacagatacttttccatcacgaggccgctcacgtaccgagccaaacgaacaacaaagagagccggtgtgatgatcggtctggcttgggtcatctcctttgtcctttgggctcctgccatcttgttctggcaatactttgttggaaagagaactgtgcctccgggagagtgcttcattcagttcctcagtgagcccaccattacttttggcacagccatcgctggtttttatatgcctgtcaccattatgactattttatactggaggatctataaggaaactgaaaagcgtaccaaagagcttgctggcctgcaagcctctgggacagaggcagagacagaaaactttgtccaccccacgggcagttctcgaagctgcagcagttacgaacttcaacagcaaagcatgaaacgctccaacaggaggaagtatggccgctgccacttctggttcacaaccaagagctggaaacccagctccgagcagatggaccaagaccacagcagcagtgacagttggaacaacaatgatgctgctgcctccctggagaactccgcctcctccgacgaggaggacattggctccgagacgagagccatctactccatcgtgctcaagcttccgggtcacagcaccatcctcaactccaccaagttaccctcatcggacaacctgcaggtgcctgaggaggagctggggatggtggacttggagaggaaagccgacaagctgcaggcccagaagagcgtggacgatggaggcagttttccaaaaagcttctccaagcttcccatccagctagagtcagccgtggacacagctaagacttctgacgtcaactcctcagtgggtaagagcacggccactctacctctgtccttcaaggaagccactctggccaagaggtttgctctgaagaccagaagtcagatcactaagcggaaaaggatgtccctggtcaaggagaagaaagcggcccagaccctcagtgcgatcttgcttgccttcatcatcacttggaccccatacaacatcatggttctggtgaacaccttttgtgacagctgcatacccaaaaccttttggaatctgggctactggctgtgctacatcaacagcaccgtgaaccccgtgtgctatgctctgtgcaacaaaacattcagaaccactttcaagatgctgctgctgtgccagtgtgacaaaaaaaagaggcgcaagcagcagtaccagcagagacagtcggtcatttttcacaagcgcgcacccgagcaggccttgaaggatcccccggtcgccaccatggtgagcaagggcgaggaggataacatggccatcatcaaggagttcatgcgcttcaaggtgcacatggagggctccgtgaacggccacgagttcgagatcgagggcgagggcgagggccgcccctacgagggcacccagaccgccaagctgaaggtgaccaagggtggccccctgcccttcgcctgggacatcctgtcccctcagttcatgtacggctccaaggcctacgtgaagcaccccgccgacatccccgactacttgaagctgtccttccccgagggcttcaagtgggagcgcgtgatgaacttcgaggacggcggcgtggtgaccgtgacccaggactcctccctgcaggacggcgagttcatctacaaggtgaagctgcgcggcaccaacttcccctccgacggccccgtaatgcagaagaagaccatgggctgggaggcctcctccgagcggatgtaccccgaggacggcgccctgaagggcgagatcaagcagaggctgaagctgaaggacggcggccactacgacgctgaggtcaagaccacctacaaggccaagaagcccgtgcagctgcccggcgcctacaacgtcaacatcaagttggacatcacctcccacaacgaggactacaccatcgtggaacagtacgaacgcgccgagggccgccactccaccggcggcatggacgagctgtacaagtaagaattcgatatcaagcttatcgataatcaacctctggattacaaaatttgtgaaagattgactggtattcttaactatgttgctccttttacgctatgtggatacgctgctttaatgcctttgtatcatgctattgcttcccgtatggctttcattttctcctccttgtataaatcctggttgctgtctctttatgaggagttgtggcccgttgtcaggcaacgtggcgtggtgtgcactgtgtttgctgacgcaacccccactggttggggcattgccaccacctgtcagctcctttccgggactttcgctttccccctccctattgccacggcggaactcatcgccgcctgccttgcccgctgctggacaggggctcggctgttgggcactgacaattccgtggtgttgtcggggaaatcatcgtcctttccttggctgctcgcctatgttgccacctggattctgcgcgggacgtccttctgctacgtcccttcggccctcaatccagcggaccttccttcccgcggcctgctgccggctctgcggcctcttccgcgtcttcgccttcgccctcagacgagtcggatctccctttgggccgcctccccgcatcgataccgagcgctgctcgagagatctacgggtggcatccctgtgacccctccccagtgcctctcctggccctggaagttgccactccagtgcccaccagccttgtcctaataaaattaagttgcatcattttgtctgactaggtgtccttctataatattatggggtggaggggggtggtatggagcaaggggcaagttgggaagacaacctgtagggcctgcggggtctattgggaaccaagctggagtgcagtggcacaatcttggctcactgcaatctccgcctcctgggttcaagcgattctcctgcctcagcctcccgagttgttgggattccaggcatgcatgaccaggctcagctaatttttgtttttttggtagagacggggtttcaccatattggccaggctggtctccaactcctaatctcaggtgatctacccaccttggcctcccaaattgctgggattacaggcgtgaaccactgctcccttccctgtcct

SEQ ID NO: 2 - DNA, 4384 bp, Artificial Sequence
  TAC-1-hM4D(Gi)-mCherry Construct
tgctgcagcaattcaaaggagaatcttgctgttcgggcagaagaaattcaatcaccttgtggagataatgaaaaagcttcatacttttaatcagatattgatcgattaccataatattctcccatagcaatagctgcaggcataagaaacggaaagaatggaagagatttttaggagaatacaaaaataaataagtatttgagacttagatactgcctttagtgacaagggtgaggatcctacacactatgttgctggtttcctagtcttcagcaagaaagtgtaggagagaagcaaaaaacgtcctgttcaacccctgctcctggatgtggcaaggaagaggagttacccggcttgaaacaaaagaaatcctaagtctgacacacaatgtcatgtttaaattcccctttctccaaaatgtaaaataaatctgcttccatcttctaaaatactatgggactaaacatccttttgttatgctaaggaaaagccagtattcgcgttgatttagaagagggatgttctggttatagaacgatgctgtgtctcagaaacacttaaatactattaagctagaaatagaagggaaaataatgcttccccgcatctcccctcaagtgtagtcctctttttttagcctgatttccgacgaaatgtctgaatgcctacagttatttggccatcctgaaaagtgcaacttatcctgacgtctcgagggacggaaaagttaccgaagtccaaggaatgagtcactttgctcaaatttgatgagtaatatcaggtgtcatgaaacccagtttcgaaggagaggggagggggcgtcagatctgcagacggaagcaggccgctccggattggatggcgagacctcgattttcctaaaattgcgtcatttagaacccaattgggtccagatgttatgggcatcgacgagttaccgtctcggaaactctcaatcacgcaagcgaaaggagaggaggcggctaattaaatattgagcagaaagtcgcgtggggagaatgtcacgtgggtctggaggctcaaggaggctgggataaataccgcaaggcactgagcaggcgaaagagcgcgctcggacctccttcccggcggcagctaccgagagtgcggagcgaccagcgtgcgctcggaggaaccagagaaactcagcaccccgcgggactgtccgtcgcagtaagtgggtaccgtcgacgccaccatggccaacttcacacctgtcaatggcagctcgggcaatcagtccgtgcgcctggtcacgtcatcatcccacaatcgctatgagacggtggaaatggtcttcattgccacagtgacaggctccctgagcctggtgactgtcgtgggcaacatcctggtgatgctgtccatcaaggtcaacaggcagctgcagacagtcaacaactacttcctcttcagcctggcgtgtgctgatctcatcataggcgccttctccatgaacctctacaccgtgtacatcatcaagggctactggcccctgggcgccgtggtctgcgacctgtggctggccctggactgcgtggtgagcaacgcctccgtcatgaaccttctcatcatcagctttgaccgctacttctgcgtcaccaagcctctcacctaccctgcccggcgcaccaccaagatggcaggcctcatgattgctgctgcctgggtactgtccttcgtgctctgggcgcctgccatcttgttctggcagtttgtggtgggtaagcggacggtgcccgacaaccagtgcttcatccagttcctgtccaacccagcagtgacctttggcacagccattgctggcttctacctgcctgtggtcatcatgacggtgctgtacatccacatctccctggccagtcgcagccgagtccacaagcaccggcccgagggcccgaaggagaagaaagccaagacgctggccttcctcaagagcccactaatgaagcagagcgtcaagaagcccccgcccggggaggccgcccgggaggagctgcgcaatggcaagctggaggaggcccccccgccagcgctgccaccgccaccgcgccccgtggctgataaggacacttccaatgagtccagctcaggcagtgccacccagaacaccaaggaacgcccagccacagagctgtccaccacagaggccaccacgcccgccatgcccgcccctcccctgcagccgcgggccctcaacccagcctccagatggtccaagatccagattgtgacgaagcagacaggcaatgagtgtgtgacagccattgagattgtgcctgccacgccggctggcatgcgccctgcggccaacgtggcccgcaagttcgccagcatcgctcgcaaccaggtgcgcaagaagcggcagatggcggcccgggagcgcaaagtgacacgaacgatctttgccattctgctggccttcatcctcacctggacgccctacaacgtcatggtcctggtgaacaccttctgccagagctgcatccctgacacggtgtggtccattggctactggctctgctacgtcaacagcaccatcaaccctgcctgctatgctctgtgcaacgccacctttaaaaagaccttccggcacctgctgctgtgccagtatcggaacatcggcactgccaggcgggatccaccggtcgccaccatggtgagcaagggcgaggaggataacatggccatcatcaaggagttcatgcgcttcaaggtgcacatggagggctccgtgaacggccacgagttcgagatcgagggcgagggcgagggccgcccctacgagggcacccagaccgccaagctgaaggtgaccaagggtggccccctgcccttcgcctgggacatcctgtcccctcagttcatgtacggctccaaggcctacgtgaagcaccccgccgacatccccgactacttgaagctgtccttccccgagggcttcaagtgggagcgcgtgatgaacttcgaggacggcggcgtggtgaccgtgacccaggactcctccctgcaggacggcgagttcatctacaaggtgaagctgcgcggcaccaacttcccctccgacggccccgtaatgcagaagaagaccatgggctgggaggcctcctccgagcggatgtaccccgaggacggcgccctgaagggcgagatcaagcagaggctgaagctgaaggacggcggccactacgacgctgaggtcaagaccacctacaaggccaagaagcccgtgcagctgcccggcgcctacaacgtcaacatcaagttggacatcacctcccacaacgaggactacaccatcgtggaacagtacgaacgcgccgagggccgccactccaccggcggcatggacgagctgtacaagtaagaattcgatatccagcacagtggcggccgctcgagtctagagggcccttcgaaggtaagcctatccctaaccctctcctcggtctcgattctacgcgtaccggttaatcgataatcaacctctggattacaaaatttgtgaaagattgactggtattcttaactatgttgctccttttacgctatgtggatacgctgctttaatgcctttgtatcatgctattgcttcccgtatggctttcattttctcctccttgtataaatcctggttgctgtctctttatgaggagttgtggcccgttgtcaggcaacgtggcgtggtgtgcactgtgtttgctgacgcaacccccactggttggggcattgccaccacctgtcagctcctttccgggactttcgctttccccctccctattgccacggcggaactcatcgccgcctgccttgcccgctgctggacaggggctcggctgttgggcactgacaattccgtggtgttgtcggggaaatcatcgtcctttccttggctgctcgcctgtgttgccacctggattctgcgcgggacgtccttctgctacgtcccttcggccctcaatccagcggaccttccttcccgcggcctgctgccggctctgcggcctcttccgcgtcttcgccttcgccctcagacgagtcggatctccctttgggccgcctccccgcatcgaaacccgctgatcagccggtcatcatcaccatcaccattgagtttaaacccgctgatcagcctcgactgtgccttctagttgccagccatctgttgtttgcccctcccccgtgccttccttgaccctggaaggtgccactcccactgtcctttcctaataaaatgaggaaattgcatcgcattgtctgagtaggtgtcattctattctggggggtggggtggggcaggacagcaagggggaggattgggaagacaatagcaggcatgctggggatgcggtgggctctatgg

SEQ ID NO: 3 - DNA, 2370 bp, Artificial Sequence
  PRSx8-HA-hM3D(Gq) Construct
taaaaacgcgtataagcttccgctagacaaatgtgattacccccgctagacaaatgtgattacccgcgctagacaaatgtgattaccccgctagacaaatgtgattaccccccgctagacaaatgtgattacccccgctagacaaatgtgattacccgcgctagacaaatgtgattaccccgctagacaaatgtgattacccccgaccagggcataaatggccaggtgggaccagagagctcaccccagccgactctagaaccgggatccaccatgtacccatacgatgttccagattacgctatgaccttgcacaataacagtacaacctcgcctttgtttccaaacatcagctcctcctggatacacagcccctccgatgcagggctgcccccgggaaccgtcactcatttcggcagctacaatgtttctcgagcagctggcaatttctcctctccagacggtaccaccgatgaccctctgggaggtcataccgtctggcaagtggtcttcatcgctttcttaacgggcatcctggccttggtgaccatcatcggcaacatcctggtaattgtgtcatttaaggtcaacaagcagctgaagacggtcaacaactacttcctcttaagcctggcctgtgccgatctgattatcggggtcatttcaatgaatctgtttacgacctacatcatcatgaatcgatgggccttagggaacttggcctgtgacctctggcttgccattgactgcgtagccagcaatgcctctgttatgaatcttctggtcatcagctttgacagatacttttccatcacgaggccgctcacgtaccgagccaaacgaacaacaaagagagccggtgtgatgatcggtctggcttgggtcatctcctttgtcctttgggctcctgccatcttgttctggcaatactttgttggaaagagaactgtgcctccgggagagtgcttcattcagttcctcagtgagcccaccattacttttggcacagccatcgctggtttttatatgcctgtcaccattatgactattttatactggaggatctataaggaaactgaaaagcgtaccaaagagcttgctggcctgcaagcctctgggacagaggcagagacagaaaactttgtccaccccacgggcagttctcgaagctgcagcagttacgaacttcaacagcaaagcatgaaacgctccaacaggaggaagtatggccgctgccacttctggttcacaaccaagagctggaaacccagctccgagcagatggaccaagaccacagcagcagtgacagttggaacaacaatgatgctgctgcctccctggagaactccgcctcctccgacgaggaggacattggctccgagacgagagccatctactccatcgtgctcaagcttccgggtcacagcaccatcctcaactccaccaagttaccctcatcggacaacctgcaggtgcctgaggaggagctggggatggtggacttggagaggaaagccgacaagctgcaggcccagaagagcgtggacgatggaggcagttttccaaaaagcttctccaagcttcccatccagctagagtcagccgtggacacagctaagacttctgacgtcaactcctcagtgggtaagagcacggccactctacctctgtccttcaaggaagccactctggccaagaggtttgctctgaagaccagaagtcagatcactaagcggaaaaggatgtccctggtcaaggagaagaaagcggcccagaccctcagtgcgatcttgcttgccttcatcatcacttggaccccatacaacatcatggttctggtgaacaccttttgtgacagctgcatacccaaaaccttttggaatctgggctactggctgtgctacatcaacagcaccgtgaaccccgtgtgctatgctctgtgcaacaaaacattcagaaccactttcaagatgctgctgctgtgccagtgtgacaaaaaaaagaggcgcaagcagcagtaccagcagagacagtcggtcatttttcacaagcgcgcacccgagcaggccttgtaggcggccgtacaagtaataggaattcacgcgtggtacctctagagtcgacccgggcggccgcttcgagcagacatgataagatacattgatgagtttggacaaaccacaactagaatgcagtgaaaaaaatgctttatttgtgaaatttgtgatgctattgctttatttgtaaccattataagctgcaataaacaagttaacaacaacaattgcattcattttatgtttcaggttcagggggagatgtgggaggttttttaaagcaagtaaaacctctacaaatgtggtaaaatc

SEQ ID NO: 4 - DNA, 2030 bp, Artificial Sequence
  PRSx8-HA-hM4D(Gi) Construct
taaaaacgcgtataagcttccgctagacaaatgtgattacccccgctagacaaatgtgattacccgcgctagacaaatgtgattaccccgctagacaaatgtgattaccccccgctagacaaatgtgattacccccgctagacaaatgtgattacccgcgctagacaaatgtgattaccccgctagacaaatgtgattacccccgaccagggcataaatggccaggtgggaccagagagctcaccccagccgactctagaaccgggatccaccatgtacccatacgatgttccagattacgctatgtacccatacgatgttccagattacgctgatgccaacttcacacctgtcaatggcagctcgggcaatcagtccgtgcgcctggtcacgtcatcatcccacaatcgctatgagacggtggaaatggtcttcattgccacagtgacaggctccctgagcctggtgactgtcgtgggcaacatcctggtgatgctgtccatcaaggtcaacaggcagctgcagacagtcaacaactacttcctcttcagcctggcgtgtgctgatctcatcataggcgccttctccatgaacctctacaccgtgtacatcatcaagggctactggcccctgggcgccgtggtctgcgacctgtggctggccctggactgcgtggtgagcaacgcctccgtcatgaaccttctcatcatcagctttgaccgctacttctgcgtcaccaagcctctcacctaccctgcccggcgcaccaccaagatggcaggcctcatgattgctgctgcctgggtactgtccttcgtgctctgggcgcctgccatcttgttctggcagtttgtggtgggtaagcggacggtgcccgacaaccagtgcttcatccagttcctgtccaacccagcagtgacctttggcacagccattgctggcttctacctgcctgtggtcatcatgacggtgctgtacatccacatctccctggccagtcgcagccgagtccacaagcaccggcccgagggcccgaaggagaagaaagccaagacgctggccttcctcaagagcccactaatgaagcagagcgtcaagaagcccccgcccggggaggccgcccgggaggagctgcgcaatggcaagctggaggaggcccccccgccagcgctgccaccgccaccgcgccccgtggctgataaggacacttccaatgagtccagctcaggcagtgccacccagaacaccaaggaacgcccagccacagagctgtccaccacagaggccaccacgcccgccatgcccgcccctcccctgcagccgcgggccctcaacccagcctccagatggtccaagatccagattgtgacgaagcagacaggcaatgagtgtgtgacagccattgagattgtgcctgccacgccggctggcatgcgccctgcggccaacgtggcccgcaagttcgccagcatcgctcgcaaccaggtgcgcaagaagcggcagatggcggcccgggagcgcaaagtgacacgaacgatctttgccattctgctagccttcatcctcacctggacgccctacaacgtcatggtcctggtgaacaccttctgccagagctgcatccctgacacggtgtggtccattggctactggctctgctacgtcaacagcaccatcaaccctgcctgctatgctctgtgcaacgccacctttaaaaagaccttccggcacctgctgctgtgccagtatcggaacatcggcactgccaggtaggaattcgtcgacccgggcggccgcttcgagcagacatgataagatacattgatgagtttggacaaaccacaactagaatgcagtgaaaaaaatgctttatttgtgaaatttgtgatgctattgctttatttgtaaccattataagctgcaataaacaagttaacaacaacaattgcattcattttatgtttcaggttcagggggagatgtgggaggttttttaaagcaagtaaaacctctacaaatgtggtaaaatc

SEQ ID NO: 5 - DNA, 1077 bp, Artificial Sequence
  Pituitary Adenylate Cyclase Activating Polypeptide (PACAP) promoter.
caatcttaaattttcaattattgcagaaaacacagtgacatggtttcaatttttaaaactagtaagagccacggagagtgtgaaagtgtgtagacaggaaaggtaaagatccatctgaatactaggactaactcagaagaaaaagctttgcactgaggcagggattaagcaggttctgagcactgggacattcgtggacacagaatccaagggaagattaatatgaacagcggggtgatttagacaatgaactcccacagtaagagcaccactgccaaagcttcaaatttagaggctgtggtgaaaattaaaccagtggcaaatttcaacatttgcagcatctgcgcccaaatagttcagcaccaagagcctggacagcaccacaggctctcatcctagtctcatccatcaatctattcagagacagactgtcaacccagccagactcattagatatttactgaaaatccttataattctttcctttaaaacacaaaacgacttccatgtttagtagcctatttgaaaaagcatatgcaaggaattgagagatcaaaattaaaattattaataggagatcttgatggtgcttaaatctagagatcagagttgtcattggtgggggttgagtgaaaattaagaaaaattagggactcaataaaaacatgacttcaccattctctaaattctacgagttctttacttgtctttgagaaatcagtgaaatcgaaaaccatcaaaataattggacttcttaaaaattggattgtgtgagtgaaaggtgtttatcagaagcggatgactccggatcttatcatcctggaggactgcacagaatagttaatatgttccttgagggactaggatgctgacgtcttttactgataccggatcattacgtgactgggggagaaaaaaaaggaagtcatatcatgaataaaaatcggagtgcaacagtgcaaccaaaatattctgtacttgaaggcagaaagatgttgacaaagaggtgtctcctgaaaccacgttcggacagcttattttgttaactgcatatataaaaacgagcagaaggccagt

SEQ ID NO: 6 - DNA, 3981 bp, Artificial Sequence
  PACAP-hM3D(Gq) Construct
caatcttaaattttcaattattgcagaaaacacagtgacatggtttcaatttttaaaactagtaagagccacggagagtgtgaaagtgtgtagacaggaaaggtaaagatccatctgaatactaggactaactcagaagaaaaagctttgcactgaggcagggattaagcaggttctgagcactgggacattcgtggacacagaatccaagggaagattaatatgaacagcggggtgatttagacaatgaactcccacagtaagagcaccactgccaaagcttcaaatttagaggctgtggtgaaaattaaaccagtggcaaatttcaacatttgcagcatctgcgcccaaatagttcagcaccaagagcctggacagcaccacaggctctcatcctagtctcatccatcaatctattcagagacagactgtcaacccagccagactcattagatatttactgaaaatccttataattctttcctttaaaacacaaaacgacttccatgtttagtagcctatttgaaaaagcatatgcaaggaattgagagatcaaaattaaaattattaataggagatcttgatggtgcttaaatctagagatcagagttgtcattggtgggggttgagtgaaaattaagaaaaattagggactcaataaaaacatgacttcaccattctctaaattctacgagttctttacttgtctttgagaaatcagtgaaatcgaaaaccatcaaaataattggacttcttaaaaattggattgtgtgagtgaaaggtgtttatcagaagcggatgactccggatcttatcatcctggaggactgcacagaatagttaatatgttccttgagggactaggatgctgacgtcttttactgataccggatcattacgtgactgggggagaaaaaaaaggaagtcatatcatgaataaaaatcggagtgcaacagtgcaaccaaaatattctgtacttgaaggcagaaagatgttgacaaagaggtgtctcctgaaaccacgttcggacagcttattttgttaactgcatatataaaaacgagcagaaggccagtgtcgacgccaccatgaccttgcacaataacagtacaacctcgcctttgtttccaaacatcagctcctcctggatacacagcccctccgatgcagggctgcccccgggaaccgtcactcatttcggcagctacaatgtttctcgagcagctggcaatttctcctctccagacggtaccaccgatgaccctctgggaggtcataccgtctggcaagtggtcttcatcgctttcttaacgggcatcctggccttggtgaccatcatcggcaacatcctggtaattgtgtcatttaaggtcaacaagcagctgaagacggtcaacaactacttcctcttaagcctggcctgtgccgatctgattatcggggtcatttcaatgaatctgtttacgacctacatcatcatgaatcgatgggccttagggaacttggcctgtgacctctggcttgccattgactgcgtagccagcaatgcctctgttatgaatcttctggtcatcagctttgacagatacttttccatcacgaggccgctcacgtaccgagccaaacgaacaacaaagagagccggtgtgatgatcggtctggcttgggtcatctcctttgtcctttgggctcctgccatcttgttctggcaatactttgttggaaagagaactgtgcctccgggagagtgcttcattcagttcctcagtgagcccaccattacttttggcacagccatcgctggtttttatatgcctgtcaccattatgactattttatactggaggatctataaggaaactgaaaagcgtaccaaagagcttgctggcctgcaagcctctgggacagaggcagagacagaaaactttgtccaccccacgggcagttctcgaagctgcagcagttacgaacttcaacagcaaagcatgaaacgctccaacaggaggaagtatggccgctgccacttctggttcacaaccaagagctggaaacccagctccgagcagatggaccaagaccacagcagcagtgacagttggaacaacaatgatgctgctgcctccctggagaactccgcctcctccgacgaggaggacattggctccgagacgagagccatctactccatcgtgctcaagcttccgggtcacagcaccatcctcaactccaccaagttaccctcatcggacaacctgcaggtgcctgaggaggagctggggatggtggacttggagaggaaagccgacaagctgcaggcccagaagagcgtggacgatggaggcagttttccaaaaagcttctccaagcttcccatccagctagagtcagccgtggacacagctaagacttctgacgtcaactcctcagtgggtaagagcacggccactctacctctgtccttcaaggaagccactctggccaagaggtttgctctgaagaccagaagtcagatcactaagcggaaaaggatgtccctggtcaaggagaagaaagcggcccagaccctcagtgcgatcttgcttgccttcatcatcacttggaccccatacaacatcatggttctggtgaacaccttttgtgacagctgcatacccaaaaccttttggaatctgggctactggctgtgctacatcaacagcaccgtgaaccccgtgtgctatgctctgtgcaacaaaacattcagaaccactttcaagatgctgctgctgtgccagtgtgacaaaaaaaagaggcgcaagcagcagtaccagcagagacagtcggtcatttttcacaagcgcgcacccgagcaggccttgaagaattcgatatcaagcttatcgataatcaacctctggattacaaaatttgtgaaagattgactggtattcttaactatgttgctccttttacgctatgtggatacgctgctttaatgcctttgtatcatgctattgcttcccgtatggctttcattttctcctccttgtataaatcctggttgctgtctctttatgaggagttgtggcccgttgtcaggcaacgtggcgtggtgtgcactgtgtttgctgacgcaacccccactggttggggcattgccaccacctgtcagctcctttccgggactttcgctttccccctccctattgccacggcggaactcatcgccgcctgccttgcccgctgctggacaggggctcggctgttgggcactgacaattccgtggtgttgtcggggaaatcatcgtcctttccttggctgctcgcctatgttgccacctggattctgcgcgggacgtccttctgctacgtcccttcggccctcaatccagcggaccttccttcccgcggcctgctgccggctctgcggcctcttccgcgtcttcgccttcgccctcagacgagtcggatctccctttgggccgcctccccgcatcgataccgagcgctgctcgagagatctacgggtggcatccctgtgacccctccccagtgcctctcctggccctggaagttgccactccagtgcccaccagccttgtcctaataaaattaagttgcatcattttgtctgactaggtgtccttctataatattatggggtggaggggggtggtatggagcaaggggcaagttgggaagacaacctgtagggcctgcggggtctattgggaaccaagctggagtgcagtggcacaatcttggctcactgcaatctccgcctcctgggttcaagcgattctcctgcctcagcctcccgagttgttgggattccaggcatgcatgaccaggctcagctaatttttgtttttttggtagagacggggtttcaccatattggccaggctggtctccaactcctaatctcaggtgatctacccaccttggcctcccaaattgctgggattacaggcgtgaaccactgctcccttccctgtcct

SEQ ID NO: 7 - DNA, 2343 bp, Artificial Sequence
  PRSx8-hM3D(Gq) Construct
taaaaacgcgtataagcttccgctagacaaatgtgattacccccgctagacaaatgtgattacccgcgctagacaaatgtgattaccccgctagacaaatgtgattaccccccgctagacaaatgtgattacccccgctagacaaatgtgattacccgcgctagacaaatgtgattaccccgctagacaaatgtgattacccccgaccagggcataaatggccaggtgggaccagagagctcaccccagccgactctagaaccgggatccaccatgatgaccttgcacaataacagtacaacctcgcctttgtttccaaacatcagctcctcctggatacacagcccctccgatgcagggctgcccccgggaaccgtcactcatttcggcagctacaatgtttctcgagcagctggcaatttctcctctccagacggtaccaccgatgaccctctgggaggtcataccgtctggcaagtggtcttcatcgctttcttaacgggcatcctggccttggtgaccatcatcggcaacatcctggtaattgtgtcatttaaggtcaacaagcagctgaagacggtcaacaactacttcctcttaagcctggcctgtgccgatctgattatcggggtcatttcaatgaatctgtttacgacctacatcatcatgaatcgatgggccttagggaacttggcctgtgacctctggcttgccattgactgcgtagccagcaatgcctctgttatgaatcttctggtcatcagctttgacagatacttttccatcacgaggccgctcacgtaccgagccaaacgaacaacaaagagagccggtgtgatgatcggtctggcttgggtcatctcctttgtcctttgggctcctgccatcttgttctggcaatactttgttggaaagagaactgtgcctccgggagagtgcttcattcagttcctcagtgagcccaccattacttttggcacagccatcgctggtttttatatgcctgtcaccattatgactattttatactggaggatctataaggaaactgaaaagcgtaccaaagagcttgctggcctgcaagcctctgggacagaggcagagacagaaaactttgtccaccccacgggcagttctcgaagctgcagcagttacgaacttcaacagcaaagcatgaaacgctccaacaggaggaagtatggccgctgccacttctggttcacaaccaagagctggaaacccagctccgagcagatggaccaagaccacagcagcagtgacagttggaacaacaatgatgctgctgcctccctggagaactccgcctcctccgacgaggaggacattggctccgagacgagagccatctactccatcgtgctcaagcttccgggtcacagcaccatcctcaactccaccaagttaccctcatcggacaacctgcaggtgcctgaggaggagctggggatggtggacttggagaggaaagccgacaagctgcaggcccagaagagcgtggacgatggaggcagttttccaaaaagcttctccaagcttcccatccagctagagtcagccgtggacacagctaagacttctgacgtcaactcctcagtgggtaagagcacggccactctacctctgtccttcaaggaagccactctggccaagaggtttgctctgaagaccagaagtcagatcactaagcggaaaaggatgtccctggtcaaggagaagaaagcggcccagaccctcagtgcgatcttgcttgccttcatcatcacttggaccccatacaacatcatggttctggtgaacaccttttgtgacagctgcatacccaaaaccttttggaatctgggctactggctgtgctacatcaacagcaccgtgaaccccgtgtgctatgctctgtgcaacaaaacattcagaaccactttcaagatgctgctgctgtgccagtgtgacaaaaaaaagaggcgcaagcagcagtaccagcagagacagtcggtcatttttcacaagcgcgcacccgagcaggccttgtaggcggccgtacaagtaataggaattcacgcgtggtacctctagagtcgacccgggcggccgcttcgagcagacatgataagatacattgatgagtttggacaaaccacaactagaatgcagtgaaaaaaatgctttatttgtgaaatttgtgatgctattgctttatttgtaaccattataagctgcaataaacaagttaacaacaacaattgcattcattttatgtttcaggttcagggggagatgtgggaggttttttaaagcaagtaaaacctctacaaatgtggtaaaatc

SEQ ID NO: 8 - DNA, 2002 bp, Artificial Sequence
  PRSx8-hM4D(Gi) Construct
aaaaacgcgtataagcttccgctagacaaatgtgattacccccgctagacaaatgtgattacccgcgctagacaaatgtgattaccccgctagacaaatgtgattaccccccgctagacaaatgtgattacccccgctagacaaatgtgattacccgcgctagacaaatgtgattaccccgctagacaaatgtgattacccccgaccagggcataaatggccaggtgggaccagagagctcaccccagccgactctagaaccgggatccaccatgatgtacccatacgatgttccagattacgctgatgccaacttcacacctgtcaatggcagctcgggcaatcagtccgtgcgcctggtcacgtcatcatcccacaatcgctatgagacggtggaaatggtcttcattgccacagtgacaggctccctgagcctggtgactgtcgtgggcaacatcctggtgatgctgtccatcaaggtcaacaggcagctgcagacagtcaacaactacttcctcttcagcctggcgtgtgctgatctcatcataggcgccttctccatgaacctctacaccgtgtacatcatcaagggctactggcccctgggcgccgtggtctgcgacctgtggctggccctggactgcgtggtgagcaacgcctccgtcatgaaccttctcatcatcagctttgaccgctacttctgcgtcaccaagcctctcacctaccctgcccggcgcaccaccaagatggcaggcctcatgattgctgctgcctgggtactgtccttcgtgctctgggcgcctgccatcttgttctggcagtttgtggtgggtaagcggacggtgcccgacaaccagtgcttcatccagttcctgtccaacccagcagtgacctttggcacagccattgctggcttctacctgcctgtggtcatcatgacggtgctgtacatccacatctccctggccagtcgcagccgagtccacaagcaccggcccgagggcccgaaggagaagaaagccaagacgctggccttcctcaagagcccactaatgaagcagagcgtcaagaagcccccgcccggggaggccgcccgggaggagctgcgcaatggcaagctggaggaggcccccccgccagcgctgccaccgccaccgcgccccgtggctgataaggacacttccaatgagtccagctcaggcagtgccacccagaacaccaaggaacgcccagccacagagctgtccaccacagaggccaccacgcccgccatgcccgcccctcccctgcagccgcgggccctcaacccagcctccagatggtccaagatccagattgtgacgaagcagacaggcaatgagtgtgtgacagccattgagattgtgcctgccacgccggctggcatgcgccctgcggccaacgtggcccgcaagttcgccagcatcgctcgcaaccaggtgcgcaagaagcggcagatggcggcccgggagcgcaaagtgacacgaacgatctttgccattctgctagccttcatcctcacctggacgccctacaacgtcatggtcctggtgaacaccttctgccagagctgcatccctgacacggtgtggtccattggctactggctctgctacgtcaacagcaccatcaaccctgcctgctatgctctgtgcaacgccacctttaaaaagaccttccggcacctgctgctgtgccagtatcggaacatcggcactgccaggtaggaattcgtcgacccgggcggccgcttcgagcagacatgataagatacattgatgagtttggacaaaccacaactagaatgcagtgaaaaaaatgctttatttgtgaaatttgtgatgctattgctttatttgtaaccattataagctgcaataaacaagttaacaacaacaattgcattcattttatgtttcaggttcagggggagatgtgggaggttttttaaagcaagtaaaacctctacaaatgtggtaaaatc

SEQ ID NO: 9 - DNA, 3654 bp, Artificial Sequence
  TAC-1-hM4D(Gi) Construct
tgctgcagcaattcaaaggagaatcttgctgttcgggcagaagaaattcaatcaccttgtggagataatgaaaaagcttcatacttttaatcagatattgatcgattaccataatattctcccatagcaatagctgcaggcataagaaacggaaagaatggaagagatttttaggagaatacaaaaataaataagtatttgagacttagatactgcctttagtgacaagggtgaggatcctacacactatgttgctggtttcctagtcttcagcaagaaagtgtaggagagaagcaaaaaacgtcctgttcaacccctgctcctggatgtggcaaggaagaggagttacccggcttgaaacaaaagaaatcctaagtctgacacacaatgtcatgtttaaattcccctttctccaaaatgtaaaataaatctgcttccatcttctaaaatactatgggactaaacatccttttgttatgctaaggaaaagccagtattcgcgttgatttagaagagggatgttctggttatagaacgatgctgtgtctcagaaacacttaaatactattaagctagaaatagaagggaaaataatgcttccccgcatctcccctcaagtgtagtcctctttttttagcctgatttccgacgaaatgtctgaatgcctacagttatttggccatcctgaaaagtgcaacttatcctgacgtctcgagggacggaaaagttaccgaagtccaaggaatgagtcactttgctcaaatttgatgagtaatatcaggtgtcatgaaacccagtttcgaaggagaggggagggggcgtcagatctgcagacggaagcaggccgctccggattggatggcgagacctcgattttcctaaaattgcgtcatttagaacccaattgggtccagatgttatgggcatcgacgagttaccgtctcggaaactctcaatcacgcaagcgaaaggagaggaggcggctaattaaatattgagcagaaagtcgcgtggggagaatgtcacgtgggtctggaggctcaaggaggctgggataaataccgcaaggcactgagcaggcgaaagagcgcgctcggacctccttcccggcggcagctaccgagagtgcggagcgaccagcgtgcgctcggaggaaccagagaaactcagcaccccgcgggactgtccgtcgcagtaagtgggtaccgtcgacgccaccatggccaacttcacacctgtcaatggcagctcgggcaatcagtccgtgcgcctggtcacgtcatcatcccacaatcgctatgagacggtggaaatggtcttcattgccacagtgacaggctccctgagcctggtgactgtcgtgggcaacatcctggtgatgctgtccatcaaggtcaacaggcagctgcagacagtcaacaactacttcctcttcagcctggcgtgtgctgatctcatcataggcgccttctccatgaacctctacaccgtgtacatcatcaagggctactggcccctgggcgccgtggtctgcgacctgtggctggccctggactgcgtggtgagcaacgcctccgtcatgaaccttctcatcatcagctttgaccgctacttctgcgtcaccaagcctctcacctaccctgcccggcgcaccaccaagatggcaggcctcatgattgctgctgcctgggtactgtccttcgtgctctgggcgcctgccatcttgttctggcagtttgtggtgggtaagcggacggtgcccgacaaccagtgcttcatccagttcctgtccaacccagcagtgacctttggcacagccattgctggcttctacctgcctgtggtcatcatgacggtgctgtacatccacatctccctggccagtcgcagccgagtccacaagcaccggcccgagggcccgaaggagaagaaagccaagacgctggccttcctcaagagcccactaatgaagcagagcgtcaagaagcccccgcccggggaggccgcccgggaggagctgcgcaatggcaagctggaggaggcccccccgccagcgctgccaccgccaccgcgccccgtggctgataaggacacttccaatgagtccagctcaggcagtgccacccagaacaccaaggaacgcccagccacagagctgtccaccacagaggccaccacgcccgccatgcccgcccctcccctgcagccgcgggccctcaacccagcctccagatggtccaagatccagattgtgacgaagcagacaggcaatgagtgtgtgacagccattgagattgtgcctgccacgccggctggcatgcgccctgcggccaacgtggcccgcaagttcgccagcatcgctcgcaaccaggtgcgcaagaagcggcagatggcggcccgggagcgcaaagtgacacgaacgatctttgccattctgctggccttcatcctcacctggacgccctacaacgtcatggtcctggtgaacaccttctgccagagctgcatccctgacacggtgtggtccattggctactggctctgctacgtcaacagcaccatcaaccctgcctgctatgctctgtgcaacgccacctttaaaaagaccttccggcacctgctgctgtgccagtatcggaacatcggcactgccaggcggaattcgatatccagcacagtggcggccgctcgagtctagagggcccttcgaaggtaagcctatccctaaccctctcctcggtctcgattctacgcgtaccggttaatcgataatcaacctctggattacaaaatttgtgaaagattgactggtattcttaactatgttgctccttttacgctatgtggatacgctgctttaatgcctttgtatcatgctattgcttcccgtatggctttcattttctcctccttgtataaatcctggttgctgtctctttatgaggagttgtggcccgttgtcaggcaacgtggcgtggtgtgcactgtgtttgctgacgcaacccccactggttggggcattgccaccacctgtcagctcctttccgggactttcgctttccccctccctattgccacggcggaactcatcgccgcctgccttgcccgctgctggacaggggctcggctgttgggcactgacaattccgtggtgttgtcggggaaatcatcgtcctttccttggctgctcgcctgtgttgccacctggattctgcgcgggacgtccttctgctacgtcccttcggccctcaatccagcggaccttccttcccgcggcctgctgccggctctgcggcctcttccgcgtcttcgccttcgccctcagacgagtcggatctccctttgggccgcctccccgcatcgaaacccgctgatcagccggtcatcatcaccatcaccattgagtttaaacccgctgatcagcctcgactgtgccttctagttgccagccatctgttgtttgcccctcccccgtgccttccttgaccctggaaggtgccactcccactgtcctttcctaataaaatgaggaaattgcatcgcattgtctgagtaggtgtcattctattctggggggtggggtggggcaggacagcaagggggaggattgggaagacaatagcaggcatgctggggatgcggtgggctctatgg

SEQ ID NO: 10 - DNA, 4424 bp, Artificial Sequence
  TAC-1-hM3D(Gq)-mCherry Construct
tgctgcagcaattcaaaggagaatcttgctgttcgggcagaagaaattcaatcaccttgtggagataatgaaaaagcttcatacttttaatcagatattgatcgattaccataatattctcccatagcaatagctgcaggcataagaaacggaaagaatggaagagatttttaggagaatacaaaaataaataagtatttgagacttagatactgcctttagtgacaagggtgaggatcctacacactatgttgctggtttcctagtcttcagcaagaaagtgtaggagagaagcaaaaaacgtcctgttcaacccctgctcctggatgtggcaaggaagaggagttacccggcttgaaacaaaagaaatcctaagtctgacacacaatgtcatgtttaaattcccctttctccaaaatgtaaaataaatctgcttccatcttctaaaatactatgggactaaacatccttttgttatgctaaggaaaagccagtattcgcgttgatttagaagagggatgttctggttatagaacgatgctgtgtctcagaaacacttaaatactattaagctagaaatagaagggaaaataatgcttccccgcatctcccctcaagtgtagtcctctttttttagcctgatttccgacgaaatgtctgaatgcctacagttatttggccatcctgaaaagtgcaacttatcctgacgtctcgagggacggaaaagttaccgaagtccaaggaatgagtcactttgctcaaatttgatgagtaatatcaggtgtcatgaaacccagtttcgaaggagaggggagggggcgtcagatctgcagacggaagcaggccgctccggattggatggcgagacctcgattttcctaaaattgcgtcatttagaacccaattgggtccagatgttatgggcatcgacgagttaccgtctcggaaactctcaatcacgcaagcgaaaggagaggaggcggctaattaaatattgagcagaaagtcgcgtggggagaatgtcacgtgggtctggaggctcaaggaggctgggataaataccgcaaggcactgagcaggcgaaagagcgcgctcggacctccttcccggcggcagctaccgagagtgcggagcgaccagcgtgcgctcggaggaaccagagaaactcagcaccccgcgggactgtccgtcgcagtaagtgggtaccgtcgacgccaccatgaccttgcacaataacagtacaacctcgcctttgtttccaaacatcagctcctcctggatacacagcccctccgatgcagggctgcccccgggaaccgtcactcatttcggcagctacaatgtttctcgagcagctggcaatttctcctctccagacggtaccaccgatgaccctctgggaggtcataccgtctggcaagtggtcttcatcgctttcttaacgggcatcctggccttggtgaccatcatcggcaacatcctggtaattgtgtcatttaaggtcaacaagcagctgaagacggtcaacaactacttcctcttaagcctggcctgtgccgatctgattatcggggtcatttcaatgaatctgtttacgacctacatcatcatgaatcgatgggccttagggaacttggcctgtgacctctggcttgccattgactgcgtagccagcaatgcctctgttatgaatcttctggtcatcagctttgacagatacttttccatcacgaggccgctcacgtaccgagccaaacgaacaacaaagagagccggtgtgatgatcggtctggcttgggtcatctcctttgtcctttgggctcctgccatcttgttctggcaatactttgttggaaagagaactgtgcctccgggagagtgcttcattcagttcctcagtgagcccaccattacttttggcacagccatcgctggtttttatatgcctgtcaccattatgactattttatactggaggatctataaggaaactgaaaagcgtaccaaagagcttgctggcctgcaagcctctgggacagaggcagagacagaaaactttgtccaccccacgggcagttctcgaagctgcagcagttacgaacttcaacagcaaagcatgaaacgctccaacaggaggaagtatggccgctgccacttctggttcacaaccaagagctggaaacccagctccgagcagatggaccaagaccacagcagcagtgacagttggaacaacaatgatgctgctgcctccctggagaactccgcctcctccgacgaggaggacattggctccgagacgagagccatctactccatcgtgctcaagcttccgggtcacagcaccatcctcaactccaccaagttaccctcatcggacaacctgcaggtgcctgaggaggagctggggatggtggacttggagaggaaagccgacaagctgcaggcccagaagagcgtggacgatggaggcagttttccaaaaagcttctccaagcttcccatccagctagagtcagccgtggacacagctaagacttctgacgtcaactcctcagtgggtaagagcacggccactctacctctgtccttcaaggaagccactctggccaagaggtttgctctgaagaccagaagtcagatcactaagcggaaaaggatgtccctggtcaaggagaagaaagcggcccagaccctcagtgcgatcttgcttgccttcatcatcacttggaccccatacaacatcatggttctggtgaacaccttttgtgacagctgcatacccaaaaccttttggaatctgggctactggctgtgctacatcaacagcaccgtgaaccccgtgtgctatgctctgtgcaacaaaacattcagaaccactttcaagatgctgctgctgtgccagtgtgacaaaaaaaagaggcgcaagcagcagtaccagcagagacagtcggtcatttttcacaagcgcgcacccgagcaggccttgaaggatccaccggtcgccaccatggtgagcaagggcgaggaggataacatggccatcatcaaggagttcatgcgcttcaaggtgcacatggagggctccgtgaacggccacgagttcgagatcgagggcgagggcgagggccgcccctacgagggcacccagaccgccaagctgaaggtgaccaagggtggccccctgcccttcgcctgggacatcctgtcccctcagttcatgtacggctccaaggcctacgtgaagcaccccgccgacatccccgactacttgaagctgtccttccccgagggcttcaagtgggagcgcgtgatgaacttcgaggacggcggcgtggtgaccgtgacccaggactcctccctgcaggacggcgagttcatctacaaggtgaagctgcgcggcaccaacttcccctccgacggccccgtaatgcagaagaagaccatgggctgggaggcctcctccgagcggatgtaccccgaggacggcgccctgaagggcgagatcaagcagaggctgaagctgaaggacggcggccactacgacgctgaggtcaagaccacctacaaggccaagaagcccgtgcagctgcccggcgcctacaacgtcaacatcaagttggacatcacctcccacaacgaggactacaccatcgtggaacagtacgaacgcgccgagggccgccactccaccggcggcatggacgagctgtacaagtaagaattcgatatccagcacagtggcggccgctcgagtctagagggcccttcgaaggtaagcctatccctaaccctctcctcggtctcgattctacgcgtaccggttaatcgataatcaacctctggattacaaaatttgtgaaagattgactggtattcttaactatgttgctccttttacgctatgtggatacgctgctttaatgcctttgtatcatgctattgcttcccgtatggctttcattttctcctccttgtataaatcctggttgctgtctctttatgaggagttgtggcccgttgtcaggcaacgtggcgtggtgtgcactgtgtttgctgacgcaacccccactggttggggcattgccaccacctgtcagctcctttccgggactttcgctttccccctccctattgccacggcggaactcatcgccgcctgccttgcccgctgctggacaggggctcggctgttgggcactgacaattccgtggtgttgtcggggaaatcatcgtcctttccttggctgctcgcctgtgttgccacctggattctgcgcgggacgtccttctgctacgtcccttcggccctcaatccagcggaccttccttcccgcggcctgctgccggctctgcggcctcttccgcgtcttcgccttcgccctcagacgagtcggatctccctttgggccgcctccccgcat

SEQ ID NO: 11 - DNA, 4379 bp, Artificial Sequence
  PACAP-hM4D(Gi)-mCherry Construct
caatcttaaattttcaattattgcagaaaacacagtgacatggtttcaatttttaaaactagtaagagccacggagagtgtgaaagtgtgtagacaggaaaggtaaagatccatctgaatactaggactaactcagaagaaaaagctttgcactgaggcagggattaagcaggttctgagcactgggacattcgtggacacagaatccaagggaagattaatatgaacagcggggtgatttagacaatgaactcccacagtaagagcaccactgccaaagcttcaaatttagaggctgtggtgaaaattaaaccagtggcaaatttcaacatttgcagcatctgcgcccaaatagttcagcaccaagagcctggacagcaccacaggctctcatcctagtctcatccatcaatctattcagagacagactgtcaacccagccagactcattagatatttactgaaaatccttataattctttcctttaaaacacaaaacgacttccatgtttagtagcctatttgaaaaagcatatgcaaggaattgagagatcaaaattaaaattattaataggagatcttgatggtgcttaaatctagagatcagagttgtcattggtgggggttgagtgaaaattaagaaaaattagggactcaataaaaacatgacttcaccattctctaaattctacgagttctttacttgtctttgagaaatcagtgaaatcgaaaaccatcaaaataattggacttcttaaaaattggattgtgtgagtgaaaggtgtttatcagaagcggatgactccggatcttatcatcctggaggactgcacagaatagttaatatgttccttgagggactaggatgctgacgtcttttactgataccggatcattacgtgactgggggagaaaaaaaaggaagtcatatcatgaataaaaatcggagtgcaacagtgcaaccaaaatattctgtacttgaaggcagaaagatgttgacaaagaggtgtctcctgaaaccacgttcggacagcttattttgttaactgcatatataaaaacgagcagaaggccagtgtcgacgccaccatggccaacttcacacctgtcaatggcagctcgggcaatcagtccgtgcgcctggtcacgtcatcatcccacaatcgctatgagacggtggaaatggtcttcattgccacagtgacaggctccctgagcctggtgactgtcgtgggcaacatcctggtgatgctgtccatcaaggtcaacaggcagctgcagacagtcaacaactacttcctcttcagcctggcgtgtgctgatctcatcataggcgccttctccatgaacctctacaccgtgtacatcatcaagggctactggcccctgggcgccgtggtctgcgacctgtggctggccctggactgcgtggtgagcaacgcctccgtcatgaaccttctcatcatcagctttgaccgctacttctgcgtcaccaagcctctcacctaccctgcccggcgcaccaccaagatggcaggcctcatgattgctgctgcctgggtactgtccttcgtgctctgggcgcctgccatcttgttctggcagtttgtggtgggtaagcggacggtgcccgacaaccagtgcttcatccagttcctgtccaacccagcagtgacctttggcacagccattgctggcttctacctgcctgtggtcatcatgacggtgctgtacatccacatctccctggccagtcgcagccgagtccacaagcaccggcccgagggcccgaaggagaagaaagccaagacgctggccttcctcaagagcccactaatgaagcagagcgtcaagaagcccccgcccggggaggccgcccgggaggagctgcgcaatggcaagctggaggaggcccccccgccagcgctgccaccgccaccgcgccccgtggctgataaggacacttccaatgagtccagctcaggcagtgccacccagaacaccaaggaacgcccagccacagagctgtccaccacagaggccaccacgcccgccatgcccgcccctcccctgcagccgcgggccctcaacccagcctccagatggtccaagatccagattgtgacgaagcagacaggcaatgagtgtgtgacagccattgagattgtgcctgccacgccggctggcatgcgccctgcggccaacgtggcccgcaagttcgccagcatcgctcgcaaccaggtgcgcaagaagcggcagatggcggcccgggagcgcaaagtgacacgaacgatctttgccattctgctggccttcatcctcacctggacgccctacaacgtcatggtcctggtgaacaccttctgccagagctgcatccctgacacggtgtggtccattggctactggctctgctacgtcaacagcaccatcaaccctgcctgctatgctctgtgcaacgccacctttaaaaagaccttccggcacctgctgctgtgccagtatcggaacatcggcactgccaggcggggatcccccggtcgccaccatggtgagcaagggcgaggaggataacatggccatcatcaaggagttcatgcgcttcaaggtgcacatggagggctccgtgaacggccacgagttcgagatcgagggcgagggcgagggccgcccctacgagggcacccagaccgccaagctgaaggtgaccaagggtggccccctgcccttcgcctgggacatcctgtcccctcagttcatgtacggctccaaggcctacgtgaagcaccccgccgacatccccgactacttgaagctgtccttccccgagggcttcaagtgggagcgcgtgatgaacttcgaggacggcggcgtggtgaccgtgacccaggactcctccctgcaggacggcgagttcatctacaaggtgaagctgcgcggcaccaacttcccctccgacggccccgtaatgcagaagaagaccatgggctgggaggcctcctccgagcggatgtaccccgaggacggcgccctgaagggcgagatcaagcagaggctgaagctgaaggacggcggccactacgacgctgaggtcaagaccacctacaaggccaagaagcccgtgcagctgcccggcgcctacaacgtcaacatcaagttggacatcacctcccacaacgaggactacaccatcgtggaacagtacgaacgcgccgagggccgccactccaccggcggcatggacgagctgtacaagtaagaattcgatatcaagcttatcgataatcaacctctggattacaaaatttgtgaaagattgactggtattcttaactatgttgctccttttacgctatgtggatacgctgctttaatgcctttgtatcatgctattgcttcccgtatggctttcattttctcctccttgtataaatcctggttgctgtctctttatgaggagttgtggcccgttgtcaggcaacgtggcgtggtgtgcactgtgtttgctgacgcaacccccactggttggggcattgccaccacctgtcagctcctttccgggactttcgctttccccctccctattgccacggcggaactcatcgccgcctgccttgcccgctgctggacaggggctcggctgttgggcactgacaattccgtggtgttgtcggggaaatcatcgtcctttccttggctgctcgcctatgttgccacctggattctgcgcgggacgtccttctgctacgtcccttcggccctcaatccagcggaccttccttcccgcggcctgctgccggctctgcggcctcttccgcgtcttcgccttcgccctcagacgagtcggatctccctttgggccgcctccccgcatcgataccgagcgctgctcgagagatctacgggtggcatccctgtgacccctccccagtgcctctcctggccctggaagttgccactccagtgcccaccagccttgtcctaataaaattaagttgcatcattttgtctgactaggtgtccttctataatattatggggtggaggggggtggtatggagcaaggggcaagttgggaagacaacctgtagggcctgcggggtctattgggaaccaagctggagtgcagtggcacaatcttggctcactgcaatctccgcctcctgggttcaagcgattctcctgcctcagcctcccgagttgttgggattccaggcatgcatgaccaggctcagctaatttttgtttttttggtagagacggggtttcaccatattggccaggctggtctccaactcctaatctcaggtgatctacccaccttggcctcccaaattgctgggattacaggcgtgaaccactgctcccttccctgtcct